European Patent Specification EP 3 563 680 B1, published August 30, 2023. Title: Genetically Modified Major Histocompatibility Complex Mice. Applicant: Regeneron Pharmaceuticals, Inc. Application EP. The sequence listing filed with the application follows.

SEQUENCE LISTING (8 sequences)

SEQ ID NO: 1 - DNA, 200 bp, Artificial
  5' homology arm of MHC I targeting construct
ggattccccatctccacagtttcacttctgcacctaacctgggtcaggtccttctgtccggacactgttgacgcgcagtcagctcttacccccattgggtggcgcgatcacccaagaaccaatcagtgtcgccgcggacgctggatataaagtccacgcagcccgcagaactcagaagtcgcgaatcgccgacaggtgcg

SEQ ID NO: 2 - DNA, 200 bp, Artificial
  3' homology arm of MHC I targeting construct
gtaaggagagtgtgggtgcagagctggggtcagggaaagctggagctttctgcagaccctgagctgctcagggctgagagctggggtcatgaccctcaccttcatttcttgtacctgtccttcccagagcctcctccatccactgtctccaacatggcgaccgttgctgttctggttgtccttggagctgcaatagtcac

SEQ ID NO: 3 - DNA, 149 bp, Artificial
  Sequence of the chimeric human/mouse MHC I locus at the 5' junction of mouse/human sequences
agtgtcgccgcggacgctggatataaagtccacgcagcccgcagaactcagaagtcgcgaatcgccgacaggtgcgatggccgtcatggcgccccgaaccctcgtcctgctactctcgggggctctggccctgacccagacctgggcgg

SEQ ID NO: 4 - DNA, 159 bp, Artificial
  Sequence of the chimeric human/mouse MHC I locus at the 3' junction of human/mouse sequences
ggtggtgccttctggacaggagcagagatacacctgccatgtgcagcatgagggtttgcccaagcccctcaccctgagatggggtaaggagagtgtgggtgcagagctggggtcagggaaagctggagctttctgcagaccctgagctgctcagggctg

SEQ ID NO: 5 - DNA, 21 bp, Artificial
  Probe for detection of hygromycin cassette
acgagcgggttcggcccattc

SEQ ID NO: 6 - DNA, 27 bp, Artificial
  Probe for detection of human HLA-A2 alpha2-alpha3 intron
agtccttcagcctccactcaggtcagg

SEQ ID NO: 7 - DNA, 25 bp, Artificial
  Probe for detection of Human HLA-A2 alpha2 exon
taccaccagtacgcctacgacggca

SEQ ID NO: 8 - DNA, 18 bp, Artificial
  Probe for detection of human HLA-A2 alpha2-alpha3 intron
atcctgtaccagagagtg